European Patent Specification EP 3 487 517 B1, published April 5, 2023. Title: Agents and methods for the prevention or treatment of H. pylori infections. Applicant: Technische Universität München et al. The sequence listing filed with the application follows.

SEQUENCE LISTING (33 sequences)

SEQ ID NO: 1 - protein, 641 aa, Helicobacter pylori
MKKTKKTILLSLTLAASLLHAEDNGVFLSVGYQIGEAVQKVKNADKVQKLSDTYEQLSRLLTNDNGTNSKTSAQAINQAVNNLNERAKTLAGGTTNSPAYQATLLALRSVLGLWNSMGYAVICGGYTKSPGENNQKDFHYTDENGNGTTINCGGSTNSNGTHSYNGTNTLKADKNVSLSIEQYEKIHEAYQILSKALKQAGLAPLNSKGEKLEAHVTTSKYQQDNQTKTTTSVIDTTNDAQNLLTQAQTIVNTLKDYCPILIAKSSSSNGGTNNANTPSWQTAGGGKNSCATFGAEFSAASDMINNAQKIVQETQQLSANQPKNITQPHNLNLNSPSSLTALAQKMLKNAQSQAEILKLANQVESDFNKLSSGHLKDYIGKCDASAISSANMTMQNQKNNWGNGCAGVEETQSLLKTSAADFNNQTPQINQAQNLANTLIQELGNNPFRNMGMIASSTTNNGALNGLGVQVGYKQFFGEKKRWGLRYYGFFDYNHAYIKSNFFNSASDVWTYGVGSDLLFNFINDKNTNFLGKNNKISFGLFGGIALAGTSWLNSQFVNLKTISNVYSAKVNTANFQFLFNLGLRTNLARPKKKDSHHAAQHGMELGVKIPTINTNYYSFLDTKLEYRRLYSVYLNYVFAY

SEQ ID NO: 2 - DNA, 1926 bp, Helicobacter pylori
atgaaaaaaacgaaaaaaacaattttgctttctctaactcttgcggcatcactcttgcatgctgaagacaacggcgtttttttaagcgtgggttatcaaatcggtgaagcggttcaaaaagtgaaaaacgccgacaaggtgcaaaaactttcagacacttatgaacaattaagccggcttttaaccaacgataatggcacaaactcaaagacaagcgcgcaagcgatcaaccaagcggttaataatttgaacgaacgcgcaaaaactttagccggtgggacaaccaattcccctgcctatcaagccacgcttttagcgttgagatcggtgttagggctatggaatagcatgggttatgcggtcatatgcggaggctataccaaaagtccaggcgaaaacaatcaaaaagatttccactacaccgatgagaatggcaacggcactacaatcaattgcggtgggagcacaaatagtaatggcactcatagttataatggcacaaatacattaaaagcagacaaaaatgtttctctatctattgagcaatatgaaaaaatccatgaagcttatcagattctttcaaaagctttaaaacaagctgggcttgctcctttaaatagcaaaggggaaaaattagaagcgcatgtaaccacatcaaagtatcaacaagataatcaaactaaaacgacaacttctgttattgatacgactaatgatgcgcaaaatcttttgactcaagcgcaaacgattgtcaatacccttaaagattattgccccatattgatagcgaaatcttctagtagtaatggcggaactaataacgcaaacaccccttcatggcaaacagccggtggcggcaaaaattcatgcgcgacttttggcgcggagtttagtgccgcttcagacatgattaataatgcgcaaaaaatcgttcaagaaacccaacaactcagcgccaaccaaccaaaaaatatcacacaaccccataatctcaaccttaactctcctagcagtcttacggctttagctcaaaaaatgctcaaaaacgcgcaatctcaagcagaaattttaaaactagccaatcaagtggagagcgattttaacaaactttcttcaggccatcttaaagactacatagggaaatgcgatgcgagcgctataagcagtgcgaatatgacaatgcaaaatcaaaagaacaattgggggaacgggtgtgctggcgtggaagaaactcagtctttgttaaaaacaagcgccgctgattttaacaaccaaacgcctcaaatcaatcaagcacaaaacctagccaacacccttattcaagaacttggcaacaacccttttaggaatatgggcatgatcgcttcttcaaccacgaataacggcgccttgaatggtcttggggtgcaagtgggttataagcaattttttggagaaaagaaaagatgggggttaaggtattatggtttctttgattacaaccacgcctacatcaaatccaatttctttaactcggcttctgatgtgtggacttatggggtgggtagcgatttgttgtttaatttcatcaacgataaaaacaccaactttttaggcaagaataacaagatttcttttgggctttttggaggcatcgccttagcagggacttcatggcttaattctcaattcgtgaatttaaaaaccatcagcaatgtctatagcgctaaagtgaatacggctaatttccaatttttattcaatttgggcttgagaaccaatctcgctaggcctaagaaaaaagatagccatcatgcagctcaacatggcatggaattgggcgtgaaaatccctaccattaacacgaattactattcttttctagacaccaaactagaatatagaaggctttatagcgtgtatctcaattatgtgttcgcttattaa

SEQ ID NO: 3 - protein, 641 aa, Helicobacter pylori
MKKTKKTILLSLTLAASLLHAEDNGVFLSVGYQIGEAVQKVKNADKVQKLSDTYEQLSRLLTNDNGTNSKTSAQAINQAVNNLNERAKTLAGGTTNSPAYQATLLALRSVLGLWNSMGYAVICGGYTKSPGENNQKDFHYTDENGNGTTINCGGSTNSNGTHSSSGTNTLKADKNVSLSIEQYEKIHEAYQILSKALKQAGLAPLNSKGEKLEAHVTTSKPENNSQTKTTTSVIDTTNDAQNLLTQAQTIVNTLKDYCPMLIAKSSSESSGAATTNAPSWQTAGGGKNSCATFGAEFSAASDMINNAQKIVQETQQLSANQPKNITQPHNLNLNTPSSLTALAQKMLKNAQSQAEILKLANQVESDFNKLSSGHLKDYIGKCDASAISSANMTMQNQKNNWGNGCAGVEETLSSLKTSAADFNNQTPQINQAQNLANTLIQELGNNPFRNMGMIASSTTNNGALNGLGVQVGYKQFFGEKKRWGLRYYGFFDYNHAYIKSNFFNSASDVWTYGVGSDLLFNFINDKNTNFLGKNNKISVGFFGGIALAGTSWLNSQFVNLKTISNVYSAKVNTANFQFLFNLGLRTNLARPKKKDSHHAAQHGMELGVKIPTINTNYYSFLDTKLEYRRLYSVYLNYVFAY

SEQ ID NO: 4 - DNA, 1926 bp, Helicobacter pylori
atgaaaaaaacgaaaaaaacgattctgctttctctaactctcgcggcgtcattgctccatgctgaagacaacggcgtttttttaagcgtgggttatcaaatcggtgaagcggttcaaaaagtgaaaaacgccgacaaggtgcaaaaactttcagacacttatgaacaattaagccggcttttaaccaacgataatggcacaaactcaaagacaagcgcgcaagcgatcaaccaagcggttaataatttgaacgaacgcgcaaaaactttagccggtgggacaaccaattcccctgcctatcaagccacgcttttagcgttgagatcggtgttagggctatggaatagcatgggttatgcggtcatatgcggaggttataccaaaagtccaggcgaaaacaatcaaaaagatttccactacaccgatgagaatggcaatggcactacaatcaattgcggtgggagcacaaatagtaatggcactcatagttctagtggcacaaatacattaaaagcagacaaaaatgtttctctatctattgagcaatatgaaaaaatccatgaagcttatcagattctttcaaaagctttaaaacaagccgggcttgctcctttaaatagcaaaggggaaaagttagaagcgcatgtaaccacatcaaaaccagaaaataatagtcaaactaaaacgacaacttctgttattgatacgactaatgatgcgcaaaatcttttgactcaagcgcaaacgattgtcaatacccttaaagattattgccccatgttgatagcgaaatctagtagtgaaagtagtggcgcagctactacaaacgccccttcatggcaaacagccggtggcggcaaaaattcatgtgcgacttttggtgcggagtttagtgccgcttcagacatgattaataatgcgcaaaaaatcgttcaagaaacccaacaactcagcgccaaccaaccaaaaaatatcacacaaccccataatctcaaccttaacacccctagcagtcttacggctttagctcaaaaaatgctcaaaaatgcgcaatctcaagcagaaattttaaaactagccaatcaagtggagagcgattttaacaaactttcttcaggccatcttaaagactacatagggaaatgcgatgcgagcgctataagcagtgcgaatatgacaatgcaaaatcaaaagaacaattgggggaacgggtgtgctggcgtggaagaaactctgtcttcattaaaaacaagtgccgctgattttaacaaccaaacgccacaaatcaatcaagcgcaaaacctagccaacacccttattcaagaacttggcaacaacccttttaggaatatgggcatgatcgcttcttcaaccacgaataacggcgccttgaatggccttggggtgcaagtgggttataagcaattttttggggaaaagaaaagatgggggttaaggtattatggtttctttgattacaaccacgcctatatcaaatccaatttctttaactcggcttctgatgtgtggacttatggggtgggcagcgatttattgtttaatttcatcaatgataaaaacaccaactttttaggcaagaataacaagatttcagtgggattttttggaggtatcgccttagcagggacttcatggcttaattctcaattcgtgaatttaaaaaccatcagcaatgtttatagcgctaaagtgaatacggctaacttccaatttttattcaatttgggcttgagaaccaatctcgctagacctaagaaaaaagatagtcatcatgcggctcaacatggcatggaattgggcgtgaaaatccctaccattaacacgaattattattcttttctagacactaaactagaatatcgaaggctttatagcgtgtatctcaattatgtgtttgcctattaa

SEQ ID NO: 5 - protein, 632 aa, Helicobacter pylori
MKKTKKTILLSLTLASSLLHAEDNGVFLSVGYQIGEAVQKVKNADKVQKLSDAYENLNKLLANHSHSNPEAINANSATAINQAIGNLNANTQNLIDKTDNSPAYQATLLALKSTVGLWNSIAYAVICGGYTDKPNHNTTETFYNQPGQGSDSITCGGHVGLLQAGKNNSLSIEQFATLNKAYQIIQAALKQGLPALSDTKKTVEVTIKTATNANNINVNNNNNNAADTTVSITDTFINDAQNLLTQAQTIINTLQDNCPQLKGKSSSNGGTNGANTPSWQTGANQNSCSVFGTEFSAISDMISNAQNIVQETQQLNTTPLKSIAQPNNFNLNSPNSIALAQSMLKNAQSQAAVLKLANQVGSDFNRISTGVLKNYIEECNANASSESVSSNTWGKGCAGVKQTLTSLENSNASFSSQTPQINQAQNLANTIVQELGHNPFKRVGIISSQTNNGAMNGLGVQVGYKQFFGEKKRWGLRYYGFFDYNHTYIKSNFFNSASDVWTYGVGSDLLFNFINDKNTNFLGKNNQISVGLFGGIALAGTSWLNSQFVNLKTISNVYSAKVNTANFQFLFNLGLRTNLARPKKKDSHHAGQHGMELGVKIPTINTNYYSFLDTKLEYRRLYSVYLNYVFAY

SEQ ID NO: 6 - DNA, 1899 bp, Helicobacter pylori
atgaaaaaaacgaaaaaaacgattctgctttctctaactcttgcgtcatcattgctccatgctgaagacaacggcgtttttttaagcgtgggctatcaaatcggtgaagcggttcaaaaagtgaaaaacgccgacaaggtgcaaaaactttcagacgcttatgaaaacttaaacaagcttttagctaatcacagccactccaatccagaagcgattaacgcaaacagcgccacagcgatcaatcaagcgattggtaatttaaacgcaaacacgcaaaatttaattgataaaacagacaattcccctgcctatcaagccacgcttttagcgctaaaatccacggtggggttatggaatagcatagcctacgccgtcatatgcggaggctatacggataaacccaatcacaacaccacagaaactttttacaaccagccaggacaaggttcagattcaatcacttgcggtgggcatgtggggttacttcaagcaggcaaaaataattctctatccattgaacaatttgcaacgctcaataaagcgtatcaaatcatccaagccgctttgaaacaaggtctccctgctttaagcgatacaaaaaaaacggtggaagtaaccattaaaacagcaaccaacgctaacaacattaatgtcaataataacaataacaatgctgctgacactacagttagcataactgatacttttattaacgatgcacaaaaccttttaacccaagcgcaaaccatcatcaacacccttcaagacaattgcccgcaattgaaagggaagtctagtagcaatggtggaactaatggcgcaaacaccccttcatggcaaacaggcgctaaccaaaattcgtgcagcgtttttggcacggaatttagcgctatttcagacatgattagtaacgctcaaaacatcgttcaagaaacccaacagcttaataccaccccactaaaaagcatcgcgcaacccaacaatttcaaccttaactcccctaatagtatcgctttggctcaaagcatgctcaaaaacgctcaatctcaagcagcggttttaaaactggccaatcaagtggggagcgattttaatagaatttctacaggagttcttaaaaactatatagaagaatgcaatgcgaatgcttcaagtgaaagcgtttctagtaacacttgggggaaaggctgcgcgggcgtgaaacaaactctaacttcgctagaaaatagcaacgcttctttttctagccaaacgcctcaaatcaatcaagcgcaaaacctcgctaacaccattgttcaagaactcggtcataaccctttcaaacgggtgggcatcattagctctcaaaccaataacggggcgatgaatggccttggggtgcaagtgggttataagcaattttttggagaaaagaaaagatgggggttaaggtattatggtttctttgattacaaccacacctatatcaaatccaatttctttaactcggcttctgatgtgtggacttatggggtgggcagcgatttattgtttaacttcatcaacgataaaaacaccaactttttaggtaagaataaccagatttcagtggggctttttgggggaatcgccttagcagggacttcatggcttaattctcaattcgtgaatttaaaaaccatcagcaatgtctatagcgctaaagtgaatacggctaatttccaatttttattcaatttgggcttgagaaccaatctcgctagacctaagaaaaaagatagccatcatgcgggtcaacatggcatggaattgggcgtgaaaatccctaccattaacacgaattactattcttttctagacactaaactagaatataggaggctttatagcgtgtatctcaattatgtgtttgcctattaa

SEQ ID NO: 7 - protein, 12 aa, Artificial Sequence
  Targeting peptide
NWYLPWLGTNDW

SEQ ID NO: 8 - DNA, 53 bp, Artificial Sequence
  Forward primer
gtttaactttaagaaggagatatacaaatggcggttcaaaaagtgaaaaacgc

SEQ ID NO: 9 - DNA, 50 bp, Artificial Sequence
  Reverse primer
tcaagcttattaatgatgatgatgatggtgggcgccgttattcgtggttg

SEQ ID NO: 10 - DNA, 43 bp, Artificial Sequence
  Forward primer
caccatcatcatcatcattaataagcttgatccggctgctaac

SEQ ID NO: 11 - DNA, 30 bp, Artificial Sequence
  Reverse primer
gtttaactttaagaaggagatatacaaatg

SEQ ID NO: 12 - DNA, 23 bp, Artificial Sequence
  Forward primer
ggtgacgctcagaacctgctgac

SEQ ID NO: 13 - DNA, 23 bp, Artificial Sequence
  Reverse primer
accacctttagagttcagcggag

SEQ ID NO: 14 - protein, 38 aa, Artificial Sequence
  HopQ-ID+HA
EKLEAHVTTSKYQQDNQTKTTTSVIDTTNYPYDVPDYA

SEQ ID NO: 15 - protein, 641 aa, Helicobacter pylori
MKKTKKTILLSLTLASSLLHAEDNGVFLSVGYQIGEAVQKVKNADKVQKLSDTYEQLSRLLTNDNGTNSKTSAQAINQAVNNLNERAKTLAGGTTNSPAYQATLLALRSVLGLWNSMGYAVICGGYTKSPGENNQKNFHYTDENGNGTTINCGGSTNSNGTHSSNGTNTLKADKNVSLSIEQYEKIHESYQILSKALKQAGLAPLNSKGEKLEAHVTTSKYQQDSQTKTTTSVIDTTNDAQNLLTQAQTIVNTLKDYCPMLIAKSSSGSGGGAATNTPSWQTAGGGKNSCETFGAEFSAASDMINNAQKIVQETQQLSANQPKNITQPHNLNLNTPSSLTALAQKMLKNAQSQAEILKLANQVESDFNKLSSGHLKDYIGKCDMSAISSTNMTMQSQKNNWGNGCAGVEETLTSLKTSAADFNNQTPQINQAQNLANTLIQELGNNPFRNMGMIASSTTNNGALNGLGVQVGYKQFFGEKKRWGLRYYGFFDYNHAYIKSNFFNSASDVWTYGVGSDLLFNFINDKNTNFLGKNNQISFGLFGGIALAGTSWLNSQFVNLKTISNVYSAKVNTANFQFLFNLGLRTNLARPKKKDSHHAAQHGIELGVKIPTINTNYYSFLDTKLEYRRLYSVYLNYVFAY

SEQ ID NO: 16 - DNA, 1926 bp, Helicobacter pylori
atgaaaaaaacgaaaaaaacgattctgctttctctaactcttgcgtcatcattgctccatgctgaagacaacggcgtttttttaagcgtgggttatcaaattggtgaagcggttcaaaaagtgaaaaacgccgacaaggtgcaaaaactttcagacacttatgaacaattaagccggcttttaaccaacgataatggcacaaactcaaagacaagcgcgcaagcgatcaaccaagcggttaataatttgaacgaacgcgcaaaaactttagccggtgggacaaccaattcccctgcctatcaagccacgcttttagcgttaagatcggtgttagggctatggaatagcatgggttatgcggtcatatgcggaggttataccaaaagtccaggcgaaaacaatcaaaaaaatttccactacaccgatgagaatggcaacggcactacaatcaattgcggtgggagcacaaatagtaatggcactcatagttctaatggcacaaatacattaaaagcagacaaaaatgtttctctatctattgagcaatatgaaaaaatccatgaatcctatcagattctttcaaaagctttaaaacaagccgggcttgctcctttaaatagcaaaggggaaaagttagaagcgcatgtaaccacatcaaagtatcaacaagatagtcaaactaaaacgacaacttctgttattgatacgactaatgatgcgcaaaatcttttgactcaagcgcaaacgattgtcaatacccttaaagattattgccccatgttgatagcgaaatctagtagtggaagtggtggcggagctgctacaaacaccccttcatggcaaacagccggtggcggcaaaaattcatgcgagacttttggtgcggagtttagtgccgcttcagacatgattaataatgcgcaaaaaatcgttcaagaaacccaacaactcagcgccaaccaaccaaaaaatatcacacaaccccataatctcaaccttaacacccctagcagtcttacggctttagctcaaaaaatgctcaaaaacgcgcaatctcaagcagaaattttaaaactagccaatcaagtggagagcgattttaacaaactttcttcaggccatcttaaagactacatagggaaatgcgatatgagtgctataagcagtacgaatatgacaatgcaaagtcaaaagaacaattgggggaacgggtgcgctggcgtggaagaaactctaacttcattaaaaacaagcgccgctgattttaacaaccaaacgcctcaaatcaatcaagcgcaaaacctagctaacacccttattcaagaacttggcaacaacccttttaggaatatgggcatgatcgcttcttcaaccacgaataacggcgccttgaatggccttggggtgcaagtgggttataagcaattttttggagaaaagaaaagatgggggttgagatattatggtttctttgattacaaccacgcctatatcaaatccaatttctttaattcggcttctgatgtgtggacttatggggtgggtagcgatttattgtttaatttcatcaacgataaaaacaccaactttttaggcaagaataaccagatttcttttgggctttttggaggaatcgccttagcagggacttcatggcttaattctcaattcgtgaatttaaaaaccatcagcaatgtctatagcgctaaagtgaatacggctaacttccaatttttattcaatctcggcttgagaaccaatctcgctaggcctaagaaaaaagatagccatcatgcggctcaacatggcatagaattaggcgtgaaaatccctaccattaacacgaattactattcttttctagacactaaactagaatatagaaggctttatagcgtgtatctcaattatgtgttcgcgtattaa

SEQ ID NO: 17 - protein, 14 aa, Artificial Sequence
  General consensus sequence
  misc_feature (5)..(5): Xaa is Thr or Tyr or is deleted
  misc_feature (6)..(6): Xaa is Lys or Asn or is deleted
  misc_feature (7)..(7): Xaa is Ser, Lys, Asn or Thr or is deleted
  misc_feature (9)..(9): Xaa is Gly, Ser, Gln, Arg, Thr, Ile or Val or is deleted
  misc_feature (11)..(11): Xaa is Asn or Gly or is deleted
  misc_feature (12)..(12): Xaa is Asn or His or is deleted
CGGYXXXPXEXXQK

SEQ ID NO: 18 - protein, 30 aa, Artificial Sequence
  General consensus sequence
  misc_feature (4)..(4): Xaa is Ser, Gly, Asn, Thr or Phe or is deleted
  misc_feature (5)..(5): Xaa is Thr or Ile or is deleted
  misc_feature (6)..(6): Xaa is Asn, Gly or Lys or is deleted
  misc_feature (7)..(7): Xaa is Ser or Ala or is deleted
  misc_feature (8)..(8): Xaa is Asn or Asp or is deleted
  misc_feature (10)..(10): Xaa is Gln, Lys or Arg or is deleted
  misc_feature (11)..(11): Xaa is Thr, Val or Ser or is deleted
  misc_feature (12)..(12): Xaa is His, Gln or Tyr or is deleted
  misc_feature (13)..(13): Xaa is Ser or Asn or is deleted
  misc_feature (14)..(14): Xaa is Ser, Pro or Asn or is deleted
  misc_feature (15)..(15): Xaa is Asn or Ser or is deleted
  misc_feature (17)..(17): Xaa is Thr or Val
  misc_feature (18)..(18): Xaa is Asn or Ser
  misc_feature (19)..(19): Xaa is Thr, Leu or Met or is deleted
  misc_feature (21)..(21): Xaa is Lys or Pro or is deleted
  misc_feature (23)..(23): Xaa is Asp, Gly or Ala or is deleted
  misc_feature (25)..(25): Xaa is Asn or Gly or is deleted
  misc_feature (26)..(26): Xaa is Val or Ser or is deleted
CGGXXXXXGXXXXXXGXXXLXAXKXXSLSI

SEQ ID NO: 19 - protein, 33 aa, Artificial Sequence
  General consensus sequence
  misc_feature (3)..(3): Xaa is Met, Ile or Val or is deleted
  misc_feature (6)..(6): Xaa is Ala or Gly or is deleted
  misc_feature (7)..(7): Xaa is Lys or Arg or is deleted
  misc_feature (8)..(8): Xaa is Ser or Thr or is deleted
  misc_feature (9)..(9): Xaa is Ser or Thr or is deleted
  misc_feature (10)..(10): Xaa is Ser, Asn or Gly or is deleted
  misc_feature (11)..(11): Xaa is Gly, Asn, Glu, Ser or Asp or is deleted
  misc_feature (12)..(12): Xaa is Ser, Gly or Asn or is deleted
  misc_feature (13)..(13): Xaa is Ser, Met, Gly, Asn or Thr or is deleted
  misc_feature (14)..(14): Xaa is Gly, Ala, Thr, Ser, Asn or Met or is deleted
  misc_feature (15)..(15): Xaa is Gly, Asn, Thr, Ala or Val or is deleted
  misc_feature (16)..(16): Xaa is Ala, Asn, Gly or Ser or is deleted
  misc_feature (17)..(17): Xaa is Thr, Asn, Ala, Gly or Ser or is deleted
  misc_feature (18)..(18): Xaa is Thr or Ala or is deleted
  misc_feature (20)..(20): Xaa is Thr or Ala or is deleted
  misc_feature (25)..(25): Xaa is Thr or Ile or is deleted
  misc_feature (26)..(26): Xaa is Ala, Ser, Thr or Asn or is deleted
  misc_feature (27)..(27): Xaa is Gly or Ser or is deleted
  misc_feature (28)..(28): Xaa is Gly or Asn or is deleted
  misc_feature (29)..(29): Xaa is Gly, Leu or Ser or is deleted
  misc_feature (32)..(32): Xaa is Ser or Ala or is deleted
CPXLIXXXXXXXXXXXXXNXPSWQXXXXXKNXC

SEQ ID NO: 20 - protein, 41 aa, Artificial Sequence
  General consensus sequence
  misc_feature (3)..(3): Xaa is Gly or Asp or is deleted
  misc_feature (4)..(4): Xaa is His or Tyr or is deleted
  misc_feature (7)..(7): Xaa is Asp or Asn or is deleted
  misc_feature (10)..(10): Xaa is Gly or Arg or is deleted
  misc_feature (14)..(14): Xaa is Met, Ala or Val or is deleted
  misc_feature (16)..(16): Xaa is Ala or Gly or is deleted
  misc_feature (17)..(17): Xaa is Ile or Val or is deleted
  misc_feature (19)..(19): Xaa is Ser or Gly or is deleted
  misc_feature (20)..(20): Xaa is any amino acid or is deleted
  misc_feature (21)..(21): Xaa is any amino acid or is deleted
  misc_feature (22)..(22): Xaa is any amino acid or is deleted
  misc_feature (23)..(23): Xaa is Thr, Ala or Ser or is deleted
  misc_feature (26)..(26): Xaa is Thr or Ala or is deleted
  misc_feature (27)..(27): Xaa is Met, Pro, Ala or Gln or is deleted
  misc_feature (28)..(28): Xaa is Gln, Arg, Lys or His or is deleted
  misc_feature (29)..(29): Xaa is Ser or Asn or is deleted
  misc_feature (30)..(30): Xaa is Gln or Met or is deleted
  misc_feature (32)..(32): Xaa is Asn or Ser or is deleted
  misc_feature (33)..(33): Xaa is Asn or Thr or is deleted
  misc_feature (34)..(34): Xaa is Thr, Asn or Ile or is deleted
  misc_feature (37)..(37): Xaa is Asn or Lys or is deleted
SSXXLKXYIXKCDXSXXSXXXXXNMXXXXXKXXXWGXGCAG

SEQ ID NO: 21 - protein, 14 aa, Artificial Sequence
  Peptide
CGGYTKSPGENNQK

SEQ ID NO: 22 - protein, 29 aa, Artificial Sequence
  Peptide
CGGSTNSNGTHSSNGTNTLKADKNVSLSI

SEQ ID NO: 23 - protein, 30 aa, Artificial Sequence
  Consensus sequence
CGGSTNSNGQTHSSNGTNTLKADKNVSLSI

SEQ ID NO: 24 - protein, 33 aa, Artificial Sequence
  Peptide
CPMLIAKSSSGSGGGAATNTPSWQTAGGGKNSC

SEQ ID NO: 25 - protein, 33 aa, Artificial Sequence
  Consensus sequence
CPMLIAKSSSGSSGGATTNTPSWQTAGGGKNSC

SEQ ID NO: 26 - protein, 37 aa, Artificial Sequence
  Peptide
SSGHLKDYIGKCDMSAISSTNMTMQSQKNNWGNGCAG

SEQ ID NO: 27 - protein, 38 aa, Artificial Sequence
  Consensus sequence
SSGHLKDYIGKCDASAISSANMTMQNQKNNTWGNGCAG

SEQ ID NO: 28 - protein, 108 aa, Homo sapiens
QLTTESMPFNVAEGKEVLLLVHNLPQQLFGYSWYKGERVDGNRQIVGYAIGTQQATPGPANSGRETIYPNASLLIQNVTQNDTGFYTLQVIKSDLVNEEATGQFHVYP

SEQ ID NO: 29 - protein, 110 aa, Homo sapiens
KLTIESTPFNVAEGKEVLLLVHNLPQHLFGYSWYKGERVDGNRQIIGYVIGTQQATPGPAYSGREIIYPNASLLIQNIIQNDTGFYTLHVIKSDLVNEEATGQFRVYPEL

SEQ ID NO: 30 - protein, 108 aa, Homo sapiens
KLTIESTPFNVAEGKEVLLLAHNLPQNRIGYSWYKGERVDGNSLIVGYVIGTQQATPGPAYSGRETIYPNASLLIQNVTQNDTGFYTLQVIKSDLVNEEATGQFHVYP

SEQ ID NO: 31 - protein, 108 aa, Homo sapiens
QLTIEAVPSNAAEGKEVLLLVHNLPQDPRGYNWYKGETVDANRRIIGYVISNQQITPGPAYSNRETIYPNASLLMRNVTRNDTGSYTLQVIKLNLMSEEVTGQFSVHP

SEQ ID NO: 32 - protein, 99 aa, Rattus norvegicus
PPNVVEESSVLLLTHNLPQEFQVFYWYKVTTTGLNSEIARYIRSSNTSQTEPAYSGRVTIYSNGSLFFQNVNKTDEGPYTLSVIDKQFNPIQTSVQFRV

SEQ ID NO: 33 - protein, 108 aa, Mus musculus
EVTIEAVPPQVAEDNNVLLLVHNLPLALGAFAWYKGNTTAIDKEIARFVPNSNMNFTGQAYSGREIIYSNGSLLFQMITMKDMGVYTLDMTDENYRRTQATVRFHVHP